European Patent Application EP 4 813 395 A1, published September 30, 2026. Title: 嚢胞性腎疾患の予防及び／又は治療剤. Applicant: 国立大学法人東海国立大学機構. The sequence listing filed with the application follows.

SEQUENCE LISTING (6 sequences)

SEQ ID NO: 1 - RNA, 22 nt, Homo sapiens
  source 1..22: mol_type = genomic RNA
  ncRNA 1..22: ncRNA_class = miRNA
tagcttatcagactgatgttga

SEQ ID NO: 2 - DNA, 21 bp, synthetic construct
  source 1..21: mol_type = other DNA
  misc_feature 1..21: note = SNA oligonucleotide
  misc_feature 2: note = n is diaminopurine
  misc_feature 3: note = n is diaminopurine
  misc_feature 5: note = n is diaminopurine
  misc_feature 8: note = n is diaminopurine
  misc_feature 14: note = n is diaminopurine
  misc_feature 16: note = n is diaminopurine
  misc_feature 17: note = n is diaminopurine
  misc_feature 6: note = n is thiouracil
  misc_feature 12: note = n is thiouracil
  misc_feature 15: note = n is thiouracil
  misc_feature 1..21: note = Phosphorothioate linkage
cnncnncngtcngnnnngcta

SEQ ID NO: 3 - DNA, 21 bp, synthetic construct
  source 1..21: mol_type = other DNA
  misc_feature 2: note = n is diaminopurine
  misc_feature 3: note = n is diaminopurine
  misc_feature 5: note = n is diaminopurine
  misc_feature 6: note = n is thiouracil
  misc_feature 8: note = n is diaminopurine
  misc_feature 12: note = n is thiouracil
  misc_feature 14: note = n is diaminopurine
  misc_feature 15: note = n is thiouracil
  misc_feature 16: note = n is diaminopurine
  misc_feature 17: note = n is diaminopurine
  misc_feature 1..21: note = L-aTNA oligonucleotide
  misc_feature 1..21: note = Phosphorothioate linkage
cnncnncngtcngnnnngcta

SEQ ID NO: 4 - DNA, 21 bp, synthetic construct
  source 1..21: mol_type = other DNA
  misc_feature 1..21: note = Phosphorothioate linkage
  misc_feature 1..21: note = SNA oligonucleotide
tatgatgtccatgtcgtacgc

SEQ ID NO: 5 - DNA, 21 bp, synthetic construct
  source 1..21: mol_type = other DNA
  misc_feature 1..21: note = SNA oligonucleotide
  misc_feature 2: note = n is diaminopurine
  misc_feature 3: note = n is diaminopurine
  misc_feature 5: note = n is diaminopurine
  misc_feature 8: note = n is diaminopurine
  misc_feature 14: note = n is diaminopurine
  misc_feature 16: note = n is diaminopurine
  misc_feature 17: note = n is diaminopurine
  misc_feature 6: note = n is thiouracil
  misc_feature 12: note = n is thiouracil
  misc_feature 15: note = n is thiouracil
  misc_feature 1..4: note = Phosphorothioate linkage
  misc_feature 10..12: note = Phosphorothioate linkage
  misc_feature 20: note = Phosphorothioate linkage
cnncnncngtcngnnnngcta

SEQ ID NO: 6 - DNA, 21 bp, synthetic construct
  source 1..21: mol_type = other DNA
  misc_feature 2: note = n is diaminopurine
  misc_feature 3: note = n is diaminopurine
  misc_feature 5: note = n is diaminopurine
  misc_feature 8: note = n is diaminopurine
  misc_feature 14: note = n is diaminopurine
  misc_feature 16: note = n is diaminopurine
  misc_feature 17: note = n is diaminopurine
  misc_feature 6: note = n is thiouracil
  misc_feature 12: note = n is thiouracil
  misc_feature 15: note = n is thiouracil
cnncnncngtcngnnnngcta